European Patent Application EP 4 458 838 A1, published November 6, 2024. Title: Peptide having activities of skin condition improvement and uses thereof. Applicant: CAREGEN CO., LTD. The sequence listing filed with the application follows.

SEQUENCE LISTING (13 sequences)

SEQ ID NO: 1 - protein, 9 aa, Artificial Sequence
  Peptide 1
EALKYWYEN

SEQ ID NO: 2 - DNA, 20 bp, Artificial Sequence
  Col1a1_F
caccctcaagagcctgagtc

SEQ ID NO: 3 - DNA, 20 bp, Artificial Sequence
  Col1a1_R
agacggctgagtagggaaca

SEQ ID NO: 4 - DNA, 20 bp, Artificial Sequence
  Fibronectin_F
ccaggaaccgagtacaccat

SEQ ID NO: 5 - DNA, 20 bp, Artificial Sequence
  Fibronectin_R
atacccaggttgggtgatga

SEQ ID NO: 6 - DNA, 20 bp, Artificial Sequence
  Elastin_F
gcaagacctggctttggact

SEQ ID NO: 7 - DNA, 21 bp, Artificial Sequence
  Elastin_R
gggagtttctggttagggctg

SEQ ID NO: 8 - DNA, 20 bp, Artificial Sequence
  GAPDH_F
ggagccaaaagggtcatcat

SEQ ID NO: 9 - DNA, 20 bp, Artificial Sequence
  GAPDH_R
gtgatggcatggactgtggt

SEQ ID NO: 10 - DNA, 20 bp, Artificial Sequence
  SIRT1_F
tcagtggctggaacagtgag

SEQ ID NO: 11 - DNA, 20 bp, Artificial Sequence
  SIRT1_R
tctggcatgtcccactatca

SEQ ID NO: 12 - DNA, 20 bp, Artificial Sequence
  AQP3_F
ccttcttgggtgctggaata

SEQ ID NO: 13 - DNA, 20 bp, Artificial Sequence
  AQP3_R
acacgataagggaggctgtg